European Patent Application EP 4 335 450 A1, published March 13, 2024. Title: PHARMACEUTICAL COMPOSITION FOR PREVENTING OR TREATING LUNG CANCER. Applicant: CELLEMEDY CO., LTD. The sequence listing filed with the application follows.

SEQUENCE LISTING (10 sequences)

SEQ ID NO: 1 - protein, 183 aa, homo sapiens
MTTASTSQVRQNYHQDSEAAINRQINLELYASYVYLSMSYYFDRDDVALKNFAKYFLHQSHEEREHAEKLMKLQNQRGGRIFLQDIQKPDCDDWESGLNAMECALHLEKNVNQSLLELHKLATDKNDPHLCDFIETHYLNEQVKAIKELGDHVTNLRKMGAPESGLAEYLFDKHTLGDSDNES

SEQ ID NO: 2 - protein, 183 aa, Artificial Sequence
  Human Ferritin Heavy Chain mutant
MTTASTSQVRQNYHAASEAAINAQINLELYASYVYLSMSYYFDRDDVALKNFAKYFLHQSHEEREHAEKLMKLQNQRGGRIALADIQKPDCDDWESGLNAMECALHLEKNVNQSLLELHKLATDKNDPHLCDFIETHYLNEQVKAIKELGDHVTNLRKMGAPESGLAEYLFDKHTLGDSDNES

SEQ ID NO: 3 - protein, 183 aa, Artificial Sequence
  Human Ferritin Heavy Chain mutant
MTTASTSQVRQNYHAASEAAINAQINLELYASYVYLSMSYYFDRDDVALKNFAKYFLHQSHEEREHAEKLMKLQNQRGGRIALADIQKPDCDDWESGLNAMECALHLEKNVNQSLLALHALATAKNDPHLCDFIETHYLNEQVKAIKELGDHVTNLRKMGAPESGLAEYLFDKHTLGDSDNES

SEQ ID NO: 4 - protein, 12 aa, homo sapiens
GGSYGSLYAFDI

SEQ ID NO: 5 - protein, 19 aa, homo sapiens
MPSFITLASLSTWEGYFDF

SEQ ID NO: 6 - protein, 52 aa, homo sapiens
VLNWYRMSPSNQTDKLAAFPEGGGSGGGTGGGSGTYLCGAISLAPKAQIKES

SEQ ID NO: 7 - protein, 8 aa, Artificial Sequence
  linker
GGGSGGGT

SEQ ID NO: 8 - protein, 10 aa, Artificial Sequence
  linker
GGGGSGGGGT

SEQ ID NO: 9 - protein, 12 aa, Artificial Sequence
  linker
GGGSGGGTGGGS

SEQ ID NO: 10 - protein, 24 aa, Artificial Sequence
  LLC-1 neo-antigen vaccine
ELELALSPIHYSSAIPAAGSNQVT